European Patent Specification EP 4 413 161 B1, published April 15, 2026. Title: Method. Applicant: Oxford Nanopore Technologies Plc. Application EP. The sequence listing filed with the application follows.

SEQUENCE LISTING (8 sequences)

SEQ ID NO: 1 - DNA, 3587 bp, Escherichia virus Lambda
  source 1..3587: mol_type = genomic DNA
gccatcagattgtgtttgttagtcgctgccatcagattgtgtttgttagtcgctttttttttttggaattttttttttggaattttttttttgcgctaacaacctcctgccgttttgcccgtgcatatcggtcacgaacaaatctgattactaaacacagtagcctggatttgttctatcagtaatcgaccttattcctaattaaatagagcaaatccccttattgggggtaagacatgaagatgccagaaaaacatgacctgttggccgccattctcgcggcaaaggaacaaggcatcggggcaatccttgcgtttgcaatggcgtaccttcgcggcagatataatggcggtgcgtttacaaaaacagtaatcgacgcaacgatgtgcgccattatcgcctagttcattcgtgaccttctcgacttcgccggactaagtagcaatctcgcttatataacgagcgtgtttatcggctacatcggtactgactcgattggttcgcttatcaaacgcttcgctgctaaaaaagccggagtagaagatggtagaaatcaataatcaacgtaaggcgttcctcgatatgctggcgtggtcggagggaactgataacggacgtcagaaaaccagaaatcatggttatgacgtcattgtaggcggagagctatttactgattactccgatcaccctcgcaaacttgtcacgctaaacccaaaactcaaatcaacaggcgccggacgctaccagcttctttcccgttggtgggatgcctaccgcaagcagcttggcctgaaagacttctctccgaaaagtcaggacgctgtggcattgcagcagattaaggagcgtggcgctttacctatgattgatcgtggtgatatccgtcaggcaatcgaccgttgcagcaatatctgggcttcactgccgggcgctggttatggtcagttcgagcataaggctgacagcctgattgcaaaattcaaagaagcgggcggaacggtcagagagattgatgtatgagcagagtcaccgcgattatctccgctctggttatctgcatcatcgtctgcctgtcatgggctgttaatcattaccgtgataacgccattacctacaaagcccagcgcgacaaaaatgccagagaactgaagctggcgaacgcggcaattactgacatgcagatgcgtcagcgtgatgttgctgcgctcgatgcaaaatacacgaaggagttagctgatgctaaagctgaaaatgatgctctgcgtgatgatgttgccgctggtcgtcgtcggttgcacatcaaagcagtctgtcagtcagtgcgtgaagccaccaccgcctccggcgtggataatgcagcctccccccgactggcagacaccgctgaacgggattatttcaccctcagagagaggctgatcactatgcaaaaacaactggaaggaacccagaagtatattaatgagcagtgcagatagagttgcccatatcgatgggcaactcatgcaattattgtgagcaatacacacgcgcttccagcggagtataaatgcctaaagtaataaaaccgagcaatccatttacgaatgtttgctgggtttctgttttaacaacattttctgcgccgccacaaattttggctgcatcgacagttttcttctgcccaattccagaaacgaagaaatgatgggtgatggtttcctttggtgctactgctgccggtttgttttgaacagtaaacgtctgttgagcacatcctgtaataagcagggccagcgcagtagcgagtagcatttttttcatggtgttattcccgatgctttttgaagttcgcagaatcgtatgtgtagaaaattaaacaaaccctaaacaatgagttgaaatttcatattgttaatatttattaatgtatgtcaggtgcgatgaatcgtcattgtattcccggattaactatgtccacagccctgacggggaacttctctgcgggagtgtccgggaataattaaaacgatgcacacagggtttagcgcgtacacgtattgcattatgccaacgccccggtgctgacacggaagaaaccggacgttatgatttagcgtggaaagatttgtgtagtgttctgaatgctctcagtaaatagtaatgaattatcaaaggtatagtaatatcttttatgttcatggatatttgtaacccatcggaaaactcctgctttagcaagattttccctgtattgctgaaatgtgatttctcttgatttcaacctatcataggacgtttctataagatgcgtgtttcttgagaatttaacatttacaacctttttaagtccttttattaacacggtgttatcgttttctaacacgatgtgaatattatctgtggctagatagtaaatataatgtgagacgttgtgacgttttagttcagaataaaacaattcacagtctaaatcttttcgcacttgatcgaatatttctttaaaaatggcaacctgagccattggtaaaaccttccatgtgatacgagggcgcgtagtttgcattatcgtttttatcgtttcaatctggtctgacctccttgtgttttgttgatgatttatgtcaaatattaggaatgttttcacttaatagtattggttgcgtaacaaagtgcggtcctgctggcattctggagggaaatacaaccgacagatgtatgtaaggccaacgtgctcaaatcttcatacagaaagatttgaagtaatattttaaccgctagatgaagagcaagcgcatggagcgacaaaatgaataaagaacaatctgctgatgatccctccgtggatctgattcgtgtaaaaaatatgcttaatagcaccatttctatgagttaccctgatgttgtaattgcatgtatagaacataaggtgtctctggaagcattcagagcaattgaggcagcgttggtgaagcacgataataatatgaaggattattccctggtggttgactgatcaccataactgctaatcattcaaactatttagtctgtgacagagccaacacgcagtctgtcactgtcaggaaagtggtaaaactgcaactcaattactgcaatgccctcgtaattaagtgaatttacaatatcgtcctgttcggagggaagaacgcgggatgttcattcttcatcacttttaattgatgtatatgctctcttttctgacgttagtctccgacggcaggcttcaatgacccaggctgagaaattcccggaccctttttgctcaagagcgatgttaatttgttcaatcatttggttaggaaagcggatgttgcgggttgttgttctgcgggttctgttcttcgttgacatgaggttgccccgtattcagtgtcgctgatttgtattgtctgaagttgtttttacgttaagttgatgcagatcaattaatacgatacctgcgtcataattgattatttgacgtggtttgatggcctccacgcacgttgtgatatgtagatgataatcattatcactttacgggtcctttccggtgaaaaaaaaggtaccaaaaaaaacatcgtcgtgagtagtgaaccgtaagc

SEQ ID NO: 2 - DNA, 20 bp, synthetic construct
  source 1..20: mol_type = other DNA
gggtcattgaagcctgccgt

SEQ ID NO: 3 - DNA, 20 bp, synthetic construct
  source 1..20: mol_type = other DNA
ggtttcttccgtgtcagcac

SEQ ID NO: 4 - DNA, 20 bp, synthetic construct
  source 1..20: mol_type = other DNA
tcatgtcttacccccaataa

SEQ ID NO: 5 - DNA, 20 bp, synthetic construct
  source 1..20: mol_type = other DNA
aatcagcgacactgaatacg

SEQ ID NO: 6 - DNA, 23 bp, synthetic construct
  source 1..23: mol_type = other DNA
cgtgggcgtactttatggggcgg

SEQ ID NO: 7 - DNA, 23 bp, synthetic construct
  source 1..23: mol_type = other DNA
cggactgcgataataagtggtgg

SEQ ID NO: 8 - DNA, 23 bp, synthetic construct
  source 1..23: mol_type = other DNA
tgtggtagtgagatgaaaagagg